European Patent Specification EP 4 056 691 B1, published October 25, 2023. Title: Novel malate dehydrogenase variant and a method for producing L-lysine using the same. Applicant: CJ CheilJedang Corporation. The sequence listing filed with the application follows.

SEQUENCE LISTING (11 sequences)

SEQ ID NO: 1 - protein, 328 aa, Artificial Sequence
  (T272I)_Malate dehydrogenase
MNSPQNVSTKKVTVTGAAGQISYSLLWRIANGEVFGTDTPVELKLLEIPQALGGAEGVAMELLDSAFPLLRNITITADANEAFDGANAAFLVGAKPRGKGEERADLLANNGKIFGPQGKAINDNAADDIRVLVVGNPANTNALIASAAAPDVPASRFNAMMRLDHNRAISQLATKLGRGSAEFNNIVVWGNHSATQFPDITYATVGGEKVTDLVDHDWYVEEFIPRVANRGAEIIEVRGKSSAASAASSAIDHMRDWVQGTEAWSSAAIPSIGAYGIPEGIFVGLPTVSRNGEWEIVEGLEISDFQRARIDANAQELQAEREAVRDLL

SEQ ID NO: 2 - DNA, 987 bp, Artificial Sequence
  (T272I)_NCgl2297
atgaattccccgcagaacgtctccaccaagaaggtcaccgtcaccggcgcagctggtcaaatctcttattcactgttgtggcgcatcgccaacggtgaagtattcggcaccgacacccctgtagaactgaaacttctggagatccctcaggctcttggcggggcagagggtgtggctatggaacttctggattctgccttccccctcctgcgaaacatcaccatcaccgcggatgccaatgaggcattcgacggcgctaatgcggcgtttttggtcggtgcgaagcctcgcggaaaaggcgaagagcgcgcagatttgctggctaacaacggcaagattttcggacctcaaggtaaagctatcaatgacaacgccgcagatgacattcgtgtcctagttgttggaaacccagcgaacaccaacgcgttgattgcttcagctgcggccccagatgttccagcatcccgcttcaacgcaatgatgcgccttgatcacaaccgtgcgatctcccagctggccaccaagcttggccgtggatctgcggaatttaacaacattgtggtctggggaaatcactccgcaacccagttcccagacatcacctacgcaaccgttggtggagaaaaggtcactgacctggttgatcacgattggtatgtggaggagttcattcctcgcgtggctaaccgtggcgctgaaatcattgaggtccgtggaaagtcttctgcagcttctgcagcatcctctgcgattgatcacatgcgcgattgggtacagggcaccgaggcgtggtcctctgcggcaattccttccatcggtgcatacggcattcctgagggcatttttgtcggtctgccaaccgtatcccgcaacggtgagtgggaaatcgttgaaggcctggagatttccgatttccagcgcgcccgcatcgacgcgaatgctcaggaattgcaggccgagcgcgaggcagtgcgcgacttgctctaa

SEQ ID NO: 3 - protein, 328 aa, Artificial Sequence
  (WT)_Malate dehydrogenase
MNSPQNVSTKKVTVTGAAGQISYSLLWRIANGEVFGTDTPVELKLLEIPQALGGAEGVAMELLDSAFPLLRNITITADANEAFDGANAAFLVGAKPRGKGEERADLLANNGKIFGPQGKAINDNAADDIRVLVVGNPANTNALIASAAAPDVPASRFNAMMRLDHNRAISQLATKLGRGSAEFNNIVVWGNHSATQFPDITYATVGGEKVTDLVDHDWYVEEFIPRVANRGAEIIEVRGKSSAASAASSAIDHMRDWVQGTEAWSSAAIPSTGAYGIPEGIFVGLPTVSRNGEWEIVEGLEISDFQRARIDANAQELQAEREAVRDLL

SEQ ID NO: 4 - DNA, 987 bp, Artificial Sequence
  (WT)_NCgl2297
atgaattccccgcagaacgtctccaccaagaaggtcaccgtcaccggcgcagctggtcaaatctcttattcactgttgtggcgcatcgccaacggtgaagtattcggcaccgacacccctgtagaactgaaacttctggagatccctcaggctcttggcggggcagagggtgtggctatggaacttctggattctgccttccccctcctgcgaaacatcaccatcaccgcggatgccaatgaggcattcgacggcgctaatgcggcgtttttggtcggtgcgaagcctcgcggaaaaggcgaagagcgcgcagatttgctggctaacaacggcaagattttcggacctcaaggtaaagctatcaatgacaacgccgcagatgacattcgtgtcctagttgttggaaacccagcgaacaccaacgcgttgattgcttcagctgcggccccagatgttccagcatcccgcttcaacgcaatgatgcgccttgatcacaaccgtgcgatctcccagctggccaccaagcttggccgtggatctgcggaatttaacaacattgtggtctggggaaatcactccgcaacccagttcccagacatcacctacgcaaccgttggtggagaaaaggtcactgacctggttgatcacgattggtatgtggaggagttcattcctcgcgtggctaaccgtggcgctgaaatcattgaggtccgtggaaagtcttctgcagcttctgcagcatcctctgcgattgatcacatgcgcgattgggtacagggcaccgaggcgtggtcctctgcggcaattccttccaccggtgcatacggcattcctgagggcatttttgtcggtctgccaaccgtatcccgcaacggtgagtgggaaatcgttgaaggcctggagatttccgatttccagcgcgcccgcatcgacgcgaatgctcaggaattgcaggccgagcgcgaggcagtgcgcgacttgctctaa

SEQ ID NO: 5 - DNA, 35 bp, Artificial Sequence
  NCgl2297_1F
tcgagctcggtaccctttgctggctaacaacggca

SEQ ID NO: 6 - DNA, 41 bp, Artificial Sequence
  NCgl2297_2R
caggaatgccgtatgcaccgatggaaggaattgccgcagag

SEQ ID NO: 7 - DNA, 41 bp, Artificial Sequence
  NCgl2297_3F
ctctgcggcaattccttccatcggtgcatacggcattcctg

SEQ ID NO: 8 - DNA, 35 bp, Artificial Sequence
  NCgl2297_4R
ctctagaggatccccaagttctgccatgcgacgct

SEQ ID NO: 9 - DNA, 20 bp, Artificial Sequence
  NCgl2297_5F
tttgctggctaacaacggca

SEQ ID NO: 10 - DNA, 20 bp, Artificial Sequence
  NCgl2297_6R
aagttctgccatgcgacgct

SEQ ID NO: 11 - DNA, 5803 bp, Artificial Sequence
  pDCM2_plasmid
gttcgcttgctgtccataaaaccgcccagtctagctatcgccatgtaagcccactgcaagctacctgctttctctttgcgcttgcgttttcccttgtccagatagcccagtagctgacattcatccggggtcagcaccgtttctgcggactggctttctacgtgttccgcttcctttagcagcccttgcgccctgagtgcttgcggcagcgtgaagctagcttttatcgccattcgccattcaggctgcgcaactgttgggaagggcgatcggtgcgggcctcttcgctattacgccagctggcgaaagggggatgtgctgcaaggcgattaagttgggtaacgccagggttttcccagtcacgacgttgtaaaacgacggccagtgaattcgagctcggtacccggggatcctctagagtcgacctgcaggcatgcaagcttggcgtaatcatggtcatagctgtttcctgtgtgaaattgttatccgctcacaattccacacaacatacgagccggaagcataaagtgtaaagcctggggtgcctaatgagtgagctaactcacattaattgcgttgcgctcactgcccgctttccagtcgggaaacctgtcgtgccagctgcattaatgaatcggccaacgcgcggggagaggcggtttgcgtattgggcgctcttccgcttcctcgctcactgactcgctgcgctcggtcgttcggctgcggcgagcggtatcagctcactcaaaggcggtaatacggttatccacagaatcaggggataacgcaggaaagaacatgtgagcaaaaggccagcaaaaggccaggaaccgtaaaaaggccgcgttgctggcgtttttccataggctccgcccccctgacgagcatcacaaaaatcgacgctcaagtcagaggtggcgaaacccgacaggactataaagataccaggcgtttccccctggaagctccctcgtgcgctctcctgttccgaccctgccgcttaccggatacctgtccgcctttctcccttcgggaagcgtggcgctttctcaatgctcacgctgtaggtatctcagttcggtgtaggtcgttcgctccaagctgggctgtgtgcacgaaccccccgttcagcccgaccgctgcgccttatccggtaactatcgtcttgagtccaacccggtaagacacgacttatcgccactggcagcagccactggtaacaggattagcagagcgaggtatgtaggcggtgctacagagttcttgaagtggtggcctaactacggctacactagaaggacagtatttggtatctgcgctctgctgaagccagttaccttcggaaaaagagttggtagctcttgatccggcaaacaaaccaccgctggtagcggtggtttttttgtttgcaagcagcagattacgcgcagaaaaaaaggatctcaagaagatcctttgatcttttctacggggtctgacgctcagtggaacgaaaactcacgttaagggattttggtcatgagattatcaaaaaggatcttcacctagatccttttggggtgggcgaagaactccagcatgagatccccgcgctggaggatcatccagccctgatagaaacagaagccactggagcacctcaaaaacaccatcatacactaaatcagtaagttggcagcatcacccgacgcactttgcgccgaataaatacctgtgacggaagatcacttcgcagaataaataaatcctggtgtccctgttgataccgggaagccctgggccaacttttggcgaaaatgagacgttgatcggcacgtaagaggttccaactttcaccataatgaaataagatcactaccgggcgtattttttgagttatcgagattttcaggagctgatagaaacagaagccactggagcacctcaaaaacaccatcatacactaaatcagtaagttggcagcatcacccgacgcactttgcgccgaataaatacctgtgacggaagatcacttcgcagaataaataaatcctggtgtccctgttgataccgggaagccctgggccaacttttggcgaaaatgagacgttgatcggcacgtaagaggttccaactttcaccataatgaaataagatcactaccgggcgtattttttgagttatcgagattttcaggagctctttggcatcgtctctcgcctgtcccctcagttcagtaatttcctgcatttgcctgtttccagtcggtagatattccacaaaacagcagggaagcagcgcttttccgctgcataaccctgcttcggggtcattatagcgattttttcggtatatccatcctttttcgcacgatatacaggattttgccaaagggttcgtgtagactttccttggtgtatccaacggcgtcagccgggcaggataggtgaagtaggcccacccgcgagcgggtgttccttcttcactgtcccttattcgcacctggcggtgctcaacgggaatcctgctctgcgaggctggccggctaccgccggcgtaacagatgagggcaagcggatggctgatgaaaccaagccaaccaggaagggcagcccacctatcaaggtgtactgccttccagacgaacgaagagcgattgaggaaaaggcggcggcggccggcatgagcctgtcggcctacctgctggccgtcggccagggctacaaaatcacgggcgtcgtggactatgagcacgtccgcgagggcgtcccggaaaacgattccgaagcccaacctttcatagaaggcggcggtggaatcgaaatctcgtgatggcaggttgggcgtcgcttggtcggtcatttcgaaaaaggttaggaatacggttagccatttgcctgcttttatatagttcantatgggattcacctttatgttgataagaaataaaagaaaatgccaataggatatcggcattttcttttgcgtttttatttgttaactgttaattgtccttgttcaaggatgctgtctttgacaacagatgttttcttgcctttgatgttcagcaggaagctcggcgcaaacgttgattgtttgtctgcgtagaatcctctgtttgtcatatagcttgtaatcacgacattgtttcctttcgcttgaggtacagcgaagtgtgagtaagtaaaggttacatcgttaggcggatcaagatccatttttaacacaaggccagttttgttcagcggcttgtatgggccagttaaagaattagaaacataaccaagcatgtaaatatcgttagacgtaatgccgtcaatcgtcatttttgatccgcgggagtcagtgaacaggtaccatttgccgttcattttaaagacgttcgcgcgttcaatttcatctgttactgtgttagatgcaatcagcggtttcatcacttttttcagtgtgtaatcatcgtttagctcaatcataccgagagcgccgtttgctaactcagccgtgcgttttttatcgctttgcagaagtttttgactttcttgacggaagaatgatgtgcttttgccatagtatgctttgttaaataaagattcttcgccttggtagccatcttcagttccagtgtttgcttcaaatactaagtatttgtggcctttatcttctacgtagtgaggatctctcagcgtatggttgtcgcctgagctgtagttgccttcatcgatgaactgctgtacattttgatacgtttttccgtcaccgtcaaagattgatttataatcctctacaccgttgatgttcaaagagctgtctgatgctgatacgttaacttgtgcagttgtcagtgtttgtttgccgtaatgtttaccggagaaatcagtgtagaataaacggatttttccgtcagatgtaaatgtggctgaacctgaccattcttgtgtttggtcttttaggatagaatcatttgcatcgaatttgtcgctgtctttaaagacgcggccagcgtttttccagctgtcaatagaagtttcgccgactttttgatagaacatgtaaatcgatgtgtcatccgcatttttaggatctccggctaatgcaaagacgatgtggtagccgtgatagtttgcgacagtgccgtcagcgttttgtaatggccagctgtcccaaacgtccaggccttttgcagaagagatatttttaattgtggacgaatcaaattcagaaacttgatatttttcatttttttgctgttcagggatttgcagcatatcatggcgtgtaatatgggaaatgccgtatgtttccttatatggcttttggttcgtttctttcgcaaacgcttgagttgcgcctcctgccagcagtgcggtagtaaaggttaatactgttgcttgttttgcaaactttttgatgttcatcgttcatgtctccttttttatgtactgtgttagcggtctgcttcttccagccctcctgtttgaagatggcaagttagttacgcacaataaaaaaagacctaaaatatgtaaggggtgacgccaaagtatacactttgccctttacacattttaggtcttgcctgctttatcagtaacaaacccgcgcgatttacttttcgacctcattctattagactctcgtttggattgcaactggtctattttcctcttttgtttgatagaaaatcataaaaggatttgcagactacgggcctaaagaactaaaaaatctatctgtttcttttcattctctgtattttttatagtttctgttgcatgggcataaagttgcctttttaatcacaattcagaaaatatcataatatctcatttcactaaataatagtgaacggcaggtatatgtgatgggttaaaaaggatcaccccagagtcccgctcagaagaactcgtcaagaaggcgatagaaggcgatgcgctgcgaatcgggagcggcgataccgtaaagcacgaggaagcggtcagcccattcgccgccaagctcttcagcaatatcacgggtagccaacgctatgtcctgatagcggtccgccacacccagccggccacagtcgatgaatccagaaaagcggccattttccaccatgatattcggcaagcaggcatcgccatgggtcacgacgagatcctcgccgtcgggcatccgcgccttgagcctggcgaacagttcggctggcgcgagcccctgatgctcttcgtccagatcatcctgatcgacaagaccggcttccatccgagtacgtgctcgctcgatgcgatgtttcgcttggtggtcgaatgggcaggtagccggatcaagcgtatgcagccgccgcattgcatcagccatgatggatactttctcggcaggagcaaggtgagatgacaggagatcctgccccggcacttcgcccaatagcagccagtcccttcccgcttcagtgacaacgtcgagacagctgcgcaaggaacgcccgtcgtggccagccacgatagccgcgctgcctcgtcttggagttcattcagggcaccggacaggtcggtcttgacaaaaagaaccgggcgcccctgcgctgacagccggaacacggcggcatcagagcagccgattgtctgttgtgcccagtcatagccgaatagcctctccacccaagcggccggagaacctgcgtgcaatccatcttgttcaatcatgcgaaacgatcctcatcctgtctcttgatcagatcttgatcccctgcgccatcagatccttggcggcaagaaagccatccagtttactttgcagggcttcccaaccttaccagagggcgccccagctggcaattccg